European Patent Application EP 4 147 719 A1, published March 15, 2023. Title: Antibodies against a proliferating inducing ligand (APRIL). Applicant: Aduro Biotech Holdings, Europe B.V. The sequence listing filed with the application follows.

SEQUENCE LISTING (39 sequences)

SEQ ID NO: 1 - DNA, 363 bp, Mus musculus
  source 1..363: mol_type = other DNA
gaggtccagttgcagcagtctggacctgagctggtaaagcctggggcttcagtgaagatgtcctgcaaggcttctggatacacattcactagctatgtgatgcactgggtgaagcagaagcctgggcagggccttgagtggattggatatattaatccttataatgatgctcctaaatacaatgagaagttcaaaggcaaggccacagtgacttcagacaagtcctccggcacagcctacatggagctcagcagcctgacctctgaggactctgcggtctattactgtgcaaggggcttgggttacgccctttactatgctatggactactggggtcaaggaacctcagtcaccgtctcctca

SEQ ID NO: 2 - DNA, 321 bp, Mus musculus
  source 1..321: mol_type = other DNA
gacattgtgatgacccagtctcaaaaattcaagtccacatcagtaggagacagggtcagcgtcacctgcaaggccagtcagaatgtgggtaataatgtagcctggtatcaacagaaagcagggcaatctcctaaagcactgatttcctcggcatccaaccgtgacagtggagtccctgatcgcttcacaggcagtggatctgggacagatttcactctcaccatcagcaatgtgcagtctgaagacttggcagactatttctgtcagcaatataacatctatccattcacgttcggctcggggacaaagttggaaataaaa

SEQ ID NO: 3 - DNA, 366 bp, Mus musculus
  source 1..366: mol_type = other DNA
caggttactctgaaagagtctggccctgggatattgcagccctcccagaccctcagtctgacttgttctttctctgggttttcactgagcacttatggtataggagtaggctggattcgtcagccttcagggaagggtctggagtggctggcacacatttggtggaatgataataagtactataacacagccctgaagagccggctcacaatctccaaggatacctccaacaaccaggtattcctcaagatcgccagtgtggacactgcagatactgccacatactactgtgctcgaatagctgggggtaactacgactatgctatggaccactggggtcaaggaacctcagtcaccgtctcctca

SEQ ID NO: 4 - DNA, 324 bp, Mus musculus
  source 1..324: mol_type = other DNA
caaattgttctcacccagtctccagcaatcatgtctacatctcctggggagaaggtcaccttgacctgcagtgccagctcaagtgtaagttctacctacttgtactggtaccagcagaagccaggatcctcccccaaactctggatttatagcacatccaacctggcttctggagtccctgctcgcttcagtggcagtgggtctgggacctcttactctctcacaatcagcagcatggaggctgaggatgctgcctcttatttctgccatcagtggagtagttacccacctacgttcggtgctgggaccaagctggagctgaaa

SEQ ID NO: 5 - protein, 121 aa, Mus musculus
EVQLQQSGPELVKPGASVKMSCKASGYTFTSYVMHWVKQKPGQGLEWIGYINPYNDAPKYNEKFKGKATVTSDKSSGTAYMELSSLTSEDSAVYYCARGLGYALYYAMDYWGQGTSVTVSS

SEQ ID NO: 6 - protein, 107 aa, Mus musculus
DIVMTQSQKFKSTSVGDRVSVTCKASQNVGNNVAWYQQKAGQSPKALISSASNRDSGVPDRFTGSGSGTDFTLTISNVQSEDLADYFCQQYNIYPFTFGSGTELEIK

SEQ ID NO: 7 - protein, 122 aa, Mus musculus
QVTLKESGPGILQPSQTLSLTCSFSGFSLSTYGIGVGWIRQPSGKGLEWLAHIWWNDNKYYNTALKSRLTISKDTSNNQVFLKIASVDTADTATYYCARIAGGNYDYAMDHWGQGTSVTVSS

SEQ ID NO: 8 - protein, 108 aa, Mus musculus
QIVLTQSPAIMSTSPGEKVTLTCSASSSVSSTYLYWYQQKPGSSPKLWIYSTSNLASGVPARFSGSGSGTSYSLTISSMEAEDAASYFCHQWSSYPPTFGAGTKLELK

SEQ ID NO: 9 - protein, 5 aa, Mus musculus
SYVMH

SEQ ID NO: 10 - protein, 17 aa, Mus musculus
YINPYNDAPKYNEKFKG

SEQ ID NO: 11 - protein, 12 aa, Mus musculus
GLGYALYYAMDY

SEQ ID NO: 12 - protein, 11 aa, Mus musculus
KASQNVGNNVA

SEQ ID NO: 13 - protein, 7 aa, Mus musculus
SASNRDS

SEQ ID NO: 14 - protein, 9 aa, Mus musculus
QQYNIYPFT

SEQ ID NO: 15 - protein, 7 aa, Mus musculus
TYGIGVG

SEQ ID NO: 16 - protein, 16 aa, Mus musculus
HIWWNDNKYYNTALKS

SEQ ID NO: 17 - protein, 12 aa, Mus musculus
IAGGNYDYAMDH

SEQ ID NO: 18 - protein, 12 aa, Mus musculus
SASSSVSSTYLY

SEQ ID NO: 19 - protein, 7 aa, Mus musculus
STSNLAS

SEQ ID NO: 20 - protein, 9 aa, Mus musculus
HQWSSYPPT

SEQ ID NO: 21 - protein, 147 aa, Homo sapiens
RAVLTQKQKKQHSVLHLVPINATSKDDSDVTEVMWQPALRRGRGLQAQGYGVRIQDAGVYLLYSQVLFQDVTFTMGQVVSREGQGRQETLFRCIRSMPSHPDRAYNSCYSAGVFHLHQGDILSVIIPRARAKLNLSPHGTFLGFVKL

SEQ ID NO: 22 - protein, 10 aa, Homo sapiens
QKKQHSVLHL

SEQ ID NO: 23 - protein, 8 aa, Homo sapiens
ALRRGRGL

SEQ ID NO: 24 - protein, 9 aa, Homo sapiens
QAQGYGVRI

SEQ ID NO: 25 - protein, 8 aa, Homo sapiens
QDAGVYLL

SEQ ID NO: 26 - protein, 11 aa, Homo sapiens
SREGQGRQETV

SEQ ID NO: 27 - protein, 11 aa, Homo sapiens
FHLHQGDILSV

SEQ ID NO: 28 - protein, 13 aa, Homo sapiens
INATSKDDSDVTE

SEQ ID NO: 29 - protein, 11 aa, Homo sapiens
VLFQDVTFTMG

SEQ ID NO: 30 - protein, 15 aa, Homo sapiens
IRSMPSHPDRAYNSC

SEQ ID NO: 31 - protein, 9 aa, Homo sapiens
IIPRARAKL

SEQ ID NO: 32 - protein, 11 aa, Homo sapiens
NLSPHGTFLGF

SEQ ID NO: 33 - protein, 11 aa, Homo sapiens
IRSMPSHPDRA

SEQ ID NO: 34 - protein, 6 aa, Homo sapiens
SMPSHP

SEQ ID NO: 35 - protein, 4 aa, Homo sapiens
TLFR

SEQ ID NO: 36 - protein, 9 aa, Homo sapiens
QDVTFTMGQ

SEQ ID NO: 37 - protein, 5 aa, Homo sapiens
VTFTM

SEQ ID NO: 38 - protein, 9 aa, Homo sapiens
VSREGQGRQ

SEQ ID NO: 39 - protein, 6 aa, Homo sapiens
TFTMGQ